European Patent Application EP 4 155 383 A1, published March 29, 2023. Title: Composition for prevention or treatment of respiratory diseases or inflammation induced by particulate matter comprising novel lactic acid bacteria. Applicant: GREEN CROSS WellBeing Corporation. The sequence listing filed with the application follows.

SEQUENCE LISTING (3 sequences)

SEQ ID NO: 1 - RNA, 1434 nt, Lactobacillus plantarum
ggtcgtacgaactctgtgtattgattggtgcttgcatcatgatttacatttgcagtgagtggcgaactggtgagtaacacgtgggaaacctgcccagaagcgggggataacacctggaaacagatgctaataccgcataacaacttggaccgcatggtccgagtttgaaagatggcttcggctatcacttttggatggtcccgcggcgtattagctagatggtggggtaacggctcaccatggcaatgatacgtagccgacctgagagggtaatcggccacattgggactgagacacggcccaaactcctacgggaggcagcagtagggaatcttccacaatggacgaaagtctgatggagcaacgccgcgtgagtgaagaagggtttcggctcgtaaaactctgttgttgaagaagaacatatctgagagtaactgttcaggtattgacggtatttaaccagaaagccacggctaactacgtgccagcagccgcggtaatacgtaggtggcaagcgttgtccggatttattgggcgtaaagcgagcgcaggcggttttttaagtctgatgtgaaagccttcggctcaaccgaagaagtgcatcggaaactgggaaacttgagtgcagaagaggacagtggaactccatgtgtagcggtgaaatgcgtagatatatggaagaacaccagtggcgaaggcggctgtctggtctgtaactgacgctgaggctcgaaagtatgggtagcaaacaggattagataccctggtagtccataccgtaaacgatgaatgctaagtgttggagggtttccgcccttcagtgctgcagctaacgcattaagcattccgcctggggagtacggccgcaaggctgaaactcaaaggaattgacgggggcccgcacaagcggtggagcatgtggtttaattcgaagctacgcgaagaaccttaccaggtcttgacatactatgcaaatctaagagattagacgttcccttcggggacatggatacaggtggtgcatggttgtcgtcagctcgtgtcgtgagatgttgggttaagtcccgcaacgagcgcaacccttattatcagttgccagcattaagttgggcactctggtgagactgccggtgacaaaccggaggaaggtggggatgacgtcaaatcatcatgccccttatgacctgggctacacacgtgctacaatggatggtacaacgagttgcgaactcgcgagagtaagctaatctcttaaagccattctcagttcggattgtaggctgcaactcgcctacatgaagtcggaatcgctagtaatcgcggatcagcatgccgcggtgaatacgttcccgggccttgtacacaccgcccgtcacaccatgagagtttgtaacacccaaagtcggtggggtaaccttttaggaaccagccgct

SEQ ID NO: 2 - RNA, 1499 nt, Pediococcus acidilactici
ctcaggatgaacgctggcggcgtgcctaatacatgcaagtcgaacgaacttccgttaattgatcaggacgtgcttgcactgaatgagattttaacacgaagtgagtggcggacgggtgagtaacacgtgggtaacctgcccagaagcaggggataacacctggaaacagatgctaataccgtataacagagaaaaccgcctggttttcttttaaaagatggctctgctatcacttctggatggacccgcggcgcattagctagttggtgaggtaacggctcaccaaggcgatgatgcgtagccgacctgagagggtaatcggccacattgggactgagacacggcccagactcctacgggaggcagcagtagggaatcttccacaatggacgcaagtctgatggagcaacgccgcgtgagtgaagaagggtttcggctcgtaaagctctgttgttaaagaagaacgtgggtgagagtaactgttcacccagtgacggtatttaaccagaaagccacggctaactacgtgccagcagccgcggtaatacgtaggtggcaagcgttatccggatttattgggcgtaaagcgagcgcaggcggtcttttaagtctaatgtgaaagccttcggctcaaccgaagaagtgcattggaaactgggagacttgagtgcagaagaggacagtggaactccatgtgtagcggtgaaatgcgtagatatatggaagaacaccagtggcgaaggcggctgtctggtctgtaactgacgctgaggctcgaaagcatgggtagcgaacaggattagataccctggtagtccatgccgtaaacgatgattactaagtgttggagggtttccgcccttcagtgctgcagctaacgcattaagtaatccgcctggggagtacgaccgcaaggttgaaactcaaaagaattgacgggggcccgcacaagcggtggagcatgtggtttaattcgaagctacgcgaagaaccttaccaggtcttgacatcttctgccaacctaagagattaggcgttcccttcggggacagaatgacaggtggtgcatggttgtcgtcagctcgtgtcgtgagatgttgggttaagtcccgcaacgagcgcaacccttattactagttgccagcattcagttgggcactctagtgagactgccggtgacaaaccggaggaaggtggggacgacgtcaaatcatcatgccccttatgacctgggctacacacgtgctacaatggatggtacaacgagttgcgaaaccgcgaggtttagctaatctcttaaaaccattctcagttcggactgtaggctgcaactcgcctacacgaagtcggaatcgctagtaatcgcggatcagcatgccgcggtgaatacgttcccgggccttgtacacaccgcccgtcacaccatgagagtttgtaacacccaaagccggtggggtaaccttttaggagctagccgtctaaggtgggacagatgatta

SEQ ID NO: 3 - RNA, 1188 nt, Lactobacillus rhamnosus
gttgatcggccacattgggactgagacacggcccaaactcctacgggaggcagcagtagggaatcttccacaatggacgcaagtctgatggagcaacgccgcgtgagtgaagaaggctttcgggtcgtaaaactctgttgttggagaagaatggtcggcagagtaactgttgtcggcgtgacggtatccaaccagaaagccacggctaactacgtgccagcagccgcggtaatacgtaggtggcaagcgttatccggatttattgggcgtaaagcgagcgcaggcggttttttaagtctgatgtgaaagccctcggcttaaccgaggaagtgcatcggaaactgggaaacttgagtgcagaagaggacagtggaactccatgtgtagcggtgaaatgcgtagatatatggaagaacaccagtggcgaaggcggctgtctggtctgtaactgacgctgaggctcgaaagcatgggtagcgaacaggattagataccctggtagtccatgccgtaaacgatgaatgctaggtgttggagggtttccgcccttcagtgccgcagctaacgcattaagcattccgcctggggagtacgaccgcaaggttgaaactcaaaggaattgacgggggcccgcacaagcggtggagcatgtggtttaattcgaagcaacgcgaagaaccttaccaggtcttgacatcttttgatcacctgagagatcaggtttccccttcgggggcaaaatgacaggtggtgcatggttgtcgtcagctcgtgtcgtgagatgttgggttaagtcccgcaacgagcgcaacccttatgactagttgccagcatttagttgggcactctagtaagactgccggtgacaaaccggaggaaggtggggatgacgtcaaatcatcatgccccttatgacctgggctacacacgtgctacaatggatggtacaacgagttgcgagaccgcgaggtcaagctaatctcttaaagccattctcagttcggactgtaggctgcaactcgcctacacgaagtcggaatcgctagtaatcgcggatcagcacgccgcggtgaatacgttcccgggccttgtacacaccgcccgtcacaccatgagagtttgtaacacccgaagccggtggcgtaacccttttagggagcgagccgtctaaggtgggacaaatgatta